European Patent Specification EP 3 571 223 B1, published September 18, 2024. Title: ANTIBODY MOLECULE-DRUG CONJUGATES AND USES THEREOF. Applicant: VISTERRA, INC. The sequence listing filed with the application follows.

SEQUENCE LISTING (261 sequences)

SEQ ID NO: 1 - protein, 118 aa, Artificial Sequence
  source: /note="Description of Artificial Sequence: Synthetic polypeptide"
EVQLQQSGPVLVKPGASVKMSCKASGYTFTDHYINWVKQSHGKSLEWIGGIYPYHGITKYNRNFKDKATLTVDKSSSTAYMELNSLTSELSAVYYCASGGSRRYFDVWGTGTTVTVSS

SEQ ID NO: 2 - protein, 120 aa, Artificial Sequence
  source: /note="Description of Artificial Sequence: Synthetic polypeptide"
EVQLVESGGGLVQPGGSLRLSCAASGFTFSDYYMTWVRQAPGKGLEWVGLIRNKRNGDTAEYSASVKGRFTISRDDSKNSLYLQMNSLKTEDTAVYYCARQGRGYTLDYWGQGTLVTVSS

SEQ ID NO: 3 - protein, 120 aa, Artificial Sequence
  source: /note="Description of Artificial Sequence: Synthetic polypeptide"
EVQLVESGGGLVQPGGSLRLSCAASGFTFSDYWMTWVRQAPGKGLEWVGLIRAKANGDTAEYSASVKGRFTISRDDSKNSLYLQMNSLKTEDTAVYYCARQGRGYTLDYWGQGTLVTVSS

SEQ ID NO: 4 - protein, 116 aa, Artificial Sequence
  source: /note="Description of Artificial Sequence: Synthetic polypeptide"
QVQLQQPGAELVKPGASVKMSCKASGYTFTSYWITWVKQRPGQGLEWIGDIYPGSGSTNYNEKFKSKATLTVDTSSSTAYMQLSSLTSEDSAVYYCARGSYSLDYWGQGTTLTVSS

SEQ ID NO: 5 - protein, 117 aa, Artificial Sequence
  source: /note="Description of Artificial Sequence: Synthetic polypeptide"
EVQLQQSVAELVRPGASVKLSCTASGFNIKNTYMHWVKQRPEQGLEWIGRIDPANGNTKYAPKFQGKATITADTSSNTAYLQLSSLTSEDTAIYYCAPSNYHAMDYWGQGTSVTVSS

SEQ ID NO: 6 - protein, 117 aa, Artificial Sequence
  source: /note="Description of Artificial Sequence: Synthetic polypeptide"
DVQLQESGPGLVKPSQSLSLTCSVTGYSITSGYYWNWIRQFPGNKLEWMGYISYDGSNNYNPSLKNRISITRDTSKNQFFLKLNSVTTEDTATYYCARWNGNYFDYWGQGTTLTVSS

SEQ ID NO: 7 - protein, 120 aa, Artificial Sequence
  source: /note="Description of Artificial Sequence: Synthetic polypeptide"
EVQLQQSGPVLVKPGASVKMSCKASGYTFTDYYMNWVKQSHGKSLEWIGVINPYNGGTSYNQKFKGKATLTVDKSSSTAYMELNSLTSEDSAVYYCARTRQLGLRWFAYWGQGTLVTVSA

SEQ ID NO: 8 - protein, 112 aa, Artificial Sequence
  source: /note="Description of Artificial Sequence: Synthetic polypeptide"
DVVMTQTPLSLPVSLGDQASISCRSSQRLVHSNGNTYLHWYLQKPGQSPKLLIYKVSNRFSGVPDRFSGSGSGTDFTLKISRVEAEDLGVYFCSQSTHVPYTFGGGTKLEIK

SEQ ID NO: 9 - protein, 107 aa, Artificial Sequence
  source: /note="Description of Artificial Sequence: Synthetic polypeptide"
DIQMTQSPSSVSASVGDRVTITCRASQNINIWLSWYQQKPGKAPKLLIYKASNLHTGVPSRFSGSGSGTDFTLTISSLQPEDFATYYCLQGQSYPRTFGGGTKVEIK

SEQ ID NO: 10 - protein, 112 aa, Artificial Sequence
  source: /note="Description of Artificial Sequence: Synthetic polypeptide"
DIVMTQAAPSVPVTPGESVSISCRSSKSLLHSNGNTYLYWFLQRPGQSPQRLIYYMSNLASGVPDRFSGRGSGTDFTLRISRVEAEDVGVYYCMQSLEYPLTFGAGTKLELK

SEQ ID NO: 11 - protein, 112 aa, Artificial Sequence
  source: /note="Description of Artificial Sequence: Synthetic polypeptide"
DIVMTQAAPSVPVTPGESVSISCRSSKSLLHSNGNTYLYWFLQRPGQSPQLLIYRMSNLASGVPDRFSGSGSGTAFTLRISRVEAEDVGVYYCMQHLEYPYTFGGGTKLEIK

SEQ ID NO: 12 - protein, 112 aa, Artificial Sequence
  source: /note="Description of Artificial Sequence: Synthetic polypeptide"
DIVMSQSPSSLAVSAGEKVTMSCKSSQSLLNSRTRKNYLAWYQQKPGQSPKLLIYWASTRESGVPDRFTGSGSGTDFTLTISSVQAEDLAVYYCKQSYNLWTFGGGTKLEIK

SEQ ID NO: 13 - protein, 107 aa, Artificial Sequence
  source: /note="Description of Artificial Sequence: Synthetic polypeptide"
DIQMTQSPASQSASLGESVTITCLASQTIGTWLAWYQQKPGKSPQLLIYAATSLADGVPSRFSGSGSGTKFSFKISSLQAEDFVSYYCQQLYSTPWTFGGGTKLEIK

SEQ ID NO: 14 - protein, 7 aa, Artificial Sequence
  source: /note="Description of Artificial Sequence: Synthetic peptide"
GYTFTDH

SEQ ID NO: 15 - protein, 6 aa, Artificial Sequence
  source: /note="Description of Artificial Sequence: Synthetic peptide"
YPYHGI

SEQ ID NO: 16 - protein, 9 aa, Artificial Sequence
  source: /note="Description of Artificial Sequence: Synthetic peptide"
GGSRRYFDV

SEQ ID NO: 17 - protein, 5 aa, Artificial Sequence
  source: /note="Description of Artificial Sequence: Synthetic peptide"
DHYIN

SEQ ID NO: 18 - protein, 17 aa, Artificial Sequence
  source: /note="Description of Artificial Sequence: Synthetic peptide"
GIYPYHGITKYNRNFKD

SEQ ID NO: 19 - protein, 7 aa, Artificial Sequence
  source: /note="Description of Artificial Sequence: Synthetic peptide"
GFTFSDY

SEQ ID NO: 20 - protein, 8 aa, Artificial Sequence
  source: /note="Description of Artificial Sequence: Synthetic peptide"
RNKRNGDT

SEQ ID NO: 21 - protein, 9 aa, Artificial Sequence
  source: /note="Description of Artificial Sequence: Synthetic peptide"
QGRGYTLDY

SEQ ID NO: 22 - protein, 5 aa, Artificial Sequence
  source: /note="Description of Artificial Sequence: Synthetic peptide"
DYYMT

SEQ ID NO: 23 - protein, 19 aa, Artificial Sequence
  source: /note="Description of Artificial Sequence: Synthetic peptide"
LIRNKRNGDTAEYSASVKG

SEQ ID NO: 24 - protein, 19 aa, Artificial Sequence
  source: /note="Description of Artificial Sequence: Synthetic peptide"
GSGSGSGSGSGSLPETGGG

SEQ ID NO: 25 - protein, 8 aa, Artificial Sequence
  source: /note="Description of Artificial Sequence: Synthetic peptide"
RAKANGDT

SEQ ID NO: 26 - protein, 19 aa, Artificial Sequence
  source: /note="Description of Artificial Sequence: Synthetic peptide"
PGGGGSGGGGSLPETGGSG

SEQ ID NO: 27 - protein, 5 aa, Artificial Sequence
  source: /note="Description of Artificial Sequence: Synthetic peptide"
DYWMT

SEQ ID NO: 28 - protein, 19 aa, Artificial Sequence
  source: /note="Description of Artificial Sequence: Synthetic peptide"
LIRAKANGDTAEYSASVKG

SEQ ID NO: 29 - protein, 7 aa, Artificial Sequence
  source: /note="Description of Artificial Sequence: Synthetic peptide"
GYTFTSY

SEQ ID NO: 30 - protein, 6 aa, Artificial Sequence
  source: /note="Description of Artificial Sequence: Synthetic peptide"
YPGSGS

SEQ ID NO: 31 - protein, 7 aa, Artificial Sequence
  source: /note="Description of Artificial Sequence: Synthetic peptide"
GSYSLDY

SEQ ID NO: 32 - protein, 5 aa, Artificial Sequence
  source: /note="Description of Artificial Sequence: Synthetic peptide"
SYWIT

SEQ ID NO: 33 - protein, 17 aa, Artificial Sequence
  source: /note="Description of Artificial Sequence: Synthetic peptide"
DIYPGSGSTNYNEKFKS

SEQ ID NO: 34 - protein, 7 aa, Artificial Sequence
  source: /note="Description of Artificial Sequence: Synthetic peptide"
GFNIKNT

SEQ ID NO: 35 - protein, 6 aa, Artificial Sequence
  source: /note="Description of Artificial Sequence: Synthetic peptide"
DPANGN

SEQ ID NO: 36 - protein, 8 aa, Artificial Sequence
  source: /note="Description of Artificial Sequence: Synthetic peptide"
SNYHAMDY

SEQ ID NO: 37 - protein, 5 aa, Artificial Sequence
  source: /note="Description of Artificial Sequence: Synthetic peptide"
NTYMH

SEQ ID NO: 38 - protein, 17 aa, Artificial Sequence
  source: /note="Description of Artificial Sequence: Synthetic peptide"
RIDPANGNTKYAPKFQG

SEQ ID NO: 39 - protein, 8 aa, Artificial Sequence
  source: /note="Description of Artificial Sequence: Synthetic peptide"
GYSITSGY

SEQ ID NO: 40 - protein, 5 aa, Artificial Sequence
  source: /note="Description of Artificial Sequence: Synthetic peptide"
SYDGS

SEQ ID NO: 41 - protein, 8 aa, Artificial Sequence
  source: /note="Description of Artificial Sequence: Synthetic peptide"
WNGNYFDY

SEQ ID NO: 42 - protein, 6 aa, Artificial Sequence
  source: /note="Description of Artificial Sequence: Synthetic peptide"
SGYYWN

SEQ ID NO: 43 - protein, 16 aa, Artificial Sequence
  source: /note="Description of Artificial Sequence: Synthetic peptide"
YISYDGSNNYNPSLKN

SEQ ID NO: 44 - protein, 7 aa, Artificial Sequence
  source: /note="Description of Artificial Sequence: Synthetic peptide"
GYTFTDY

SEQ ID NO: 45 - protein, 6 aa, Artificial Sequence
  source: /note="Description of Artificial Sequence: Synthetic peptide"
NPYNGG

SEQ ID NO: 46 - protein, 11 aa, Artificial Sequence
  source: /note="Description of Artificial Sequence: Synthetic peptide"
TRQLGLRWFAY

SEQ ID NO: 47 - protein, 5 aa, Artificial Sequence
  source: /note="Description of Artificial Sequence: Synthetic peptide"
DYYMN

SEQ ID NO: 48 - protein, 17 aa, Artificial Sequence
  source: /note="Description of Artificial Sequence: Synthetic peptide"
VINPYNGGTSYNQKFKG

SEQ ID NO: 49 - protein, 16 aa, Artificial Sequence
  source: /note="Description of Artificial Sequence: Synthetic peptide"
RSSQRLVHSNGNTYLH

SEQ ID NO: 50 - protein, 7 aa, Artificial Sequence
  source: /note="Description of Artificial Sequence: Synthetic peptide"
KVSNRFS

SEQ ID NO: 51 - protein, 9 aa, Artificial Sequence
  source: /note="Description of Artificial Sequence: Synthetic peptide"
SQSTHVPYT

SEQ ID NO: 52 - protein, 11 aa, Artificial Sequence
  source: /note="Description of Artificial Sequence: Synthetic peptide"
RASQNINIWLS

SEQ ID NO: 53 - protein, 7 aa, Artificial Sequence
  source: /note="Description of Artificial Sequence: Synthetic peptide"
KASNLHT

SEQ ID NO: 54 - protein, 9 aa, Artificial Sequence
  source: /note="Description of Artificial Sequence: Synthetic peptide"
LQGQSYPRT

SEQ ID NO: 55 - protein, 16 aa, Artificial Sequence
  source: /note="Description of Artificial Sequence: Synthetic peptide"
RSSKSLLHSNGNTYLY

SEQ ID NO: 56 - protein, 7 aa, Artificial Sequence
  source: /note="Description of Artificial Sequence: Synthetic peptide"
YMSNLAS

SEQ ID NO: 57 - protein, 9 aa, Artificial Sequence
  source: /note="Description of Artificial Sequence: Synthetic peptide"
MQSLEYPLT

SEQ ID NO: 58 - protein, 16 aa, Artificial Sequence
  source: /note="Description of Artificial Sequence: Synthetic peptide"
RSSKSLLHSNGNTYLY

SEQ ID NO: 59 - protein, 7 aa, Artificial Sequence
  source: /note="Description of Artificial Sequence: Synthetic peptide"
RMSNLAS

SEQ ID NO: 60 - protein, 9 aa, Artificial Sequence
  source: /note="Description of Artificial Sequence: Synthetic peptide"
MQHLEYPYT

SEQ ID NO: 61 - protein, 17 aa, Artificial Sequence
  source: /note="Description of Artificial Sequence: Synthetic peptide"
KSSQSLLNSRTRKNYLA

SEQ ID NO: 62 - protein, 7 aa, Artificial Sequence
  source: /note="Description of Artificial Sequence: Synthetic peptide"
WASTRES

SEQ ID NO: 63 - protein, 8 aa, Artificial Sequence
  source: /note="Description of Artificial Sequence: Synthetic peptide"
KQSYNLWT

SEQ ID NO: 64 - protein, 11 aa, Artificial Sequence
  source: /note="Description of Artificial Sequence: Synthetic peptide"
LASQTIGTWLA

SEQ ID NO: 65 - protein, 7 aa, Artificial Sequence
  source: /note="Description of Artificial Sequence: Synthetic peptide"
AATSLAD

SEQ ID NO: 66 - protein, 9 aa, Artificial Sequence
  source: /note="Description of Artificial Sequence: Synthetic peptide"
QQLYSTPWT

SEQ ID NO: 67 - protein, 16 aa, Artificial Sequence
  source: /note="Description of Artificial Sequence: Synthetic peptide"
ALWKTLLKKVLKAAAK

SEQ ID NO: 68 - protein, 29 aa, Artificial Sequence
  source: /note="Description of Artificial Sequence: Synthetic peptide"
RGLRRLGRKIAHGVKKYGPTVLRIIRIAG

SEQ ID NO: 69 - protein, 22 aa, Artificial Sequence
  source: /note="Description of Artificial Sequence: Synthetic peptide"
GIGKFLKKAKKFGKAFVKILKK

SEQ ID NO: 70 - protein, 26 aa, Artificial Sequence
  source: /note="Description of Artificial Sequence: Synthetic peptide"
ALWKTLLKKVLKAAAKGGGGSGGGGS

SEQ ID NO: 71 - protein, 32 aa, Artificial Sequence
  source: /note="Description of Artificial Sequence: Synthetic polypeptide"
GIGKFLKKAKKFGKAFVKILKKGGGGSGGGGS

SEQ ID NO: 72 - protein, 11 aa, Artificial Sequence
  source: /note="Description of Artificial Sequence: Synthetic peptide"
KKLLKWLKKLL

SEQ ID NO: 73 - protein, 22 aa, Artificial Sequence
  source: /note="Description of Artificial Sequence: Synthetic peptide"
GIGKFLKKAKKFGKAFVKILKK

SEQ ID NO: 74 - protein, 37 aa, Artificial Sequence
  source: /note="Description of Artificial Sequence: Synthetic polypeptide"
RLGNFFRKAKKKIGRGLKKIGQKIKDFLGNLVPRTES

SEQ ID NO: 75 - protein, 32 aa, Artificial Sequence
  source: /note="Description of Artificial Sequence: Synthetic polypeptide"
GGGGSGGGGSGIGKFLKKAKKFGKAFVKILKK

SEQ ID NO: 76 - protein, 32 aa, Artificial Sequence
  source: /note="Description of Artificial Sequence: Synthetic polypeptide"
GLRKRLRKFRNKIKEKLKKIGQKIQGLLPKLA

SEQ ID NO: 77 - protein, 26 aa, Artificial Sequence
  source: /note="Description of Artificial Sequence: Synthetic peptide"
GGGGSGGGGSALWKTLLKKVLKAAAK

SEQ ID NO: 78 - protein, 26 aa, Artificial Sequence
  source: /note="Description of Artificial Sequence: Synthetic peptide"
GWKKWFNRAKKVGKTVGGLAVDHYLG

SEQ ID NO: 79 - protein, 30 aa, Artificial Sequence
  source: /note="Description of Artificial Sequence: Synthetic polypeptide"
GAFGNFLKGVAKKAGLKILSIAQCKLFGTC

SEQ ID NO: 80 - protein, 32 aa, Artificial Sequence
  source: /note="Description of Artificial Sequence: Synthetic polypeptide"
GGGRGLRRLGRKIAHGVKKYGPTVLRIIRIAG

SEQ ID NO: 81 - DNA, 354 bp, Artificial Sequence
  source: /note="Description of Artificial Sequence: Synthetic polynucleotide"
gaggtccagctgcagcagtctggacctgtgctggtgaagcctggggcttcagtgaagatgtcctgtaaggcttctggatacacattcactgaccactatataaactgggtgaagcagagccatggaaagagccttgagtggattggaggtatttatccttaccacggtattactaagtacaaccggaatttcaaggacaaggccacattgactgttgacaagtcctccagcacagcctacatggagctcaacagcctgacatctgaactctctgcagtctattactgtgcaagcgggggaagtcgccggtacttcgatgtctggggcacagggaccacggtcaccgtctcctca

SEQ ID NO: 82 - DNA, 360 bp, Artificial Sequence
  source: /note="Description of Artificial Sequence: Synthetic polynucleotide"
gaagtgcagctcgtggaatctggaggaggacttgtgcaacctggaggttccctgcgactgtcgtgtgccgcatccggtttcaccttttccgactactacatgacctgggtcagacaggcgccggggaagggactggagtgggtcggcttgatccgcaacaagaggaacggcgatactgctgaatactcggccagcgtgaaggggcggttcaccatctcgagagatgacagcaagaactccctgtacctccaaatgaactccctgaaaaccgaggacactgcggtgtactactgcgcccgccagggtcgcggctacacgctggactattggggccagggcaccctggtcactgtgtcaagc

SEQ ID NO: 83 - DNA, 360 bp, Artificial Sequence
  source: /note="Description of Artificial Sequence: Synthetic polynucleotide"
gaagtgcagctcgtggaatctggaggaggacttgtgcaacctggaggttccctgcgactgtcgtgtgccgcatccggtttcaccttttccgactactggatgacctgggtcagacaggcgccggggaagggactggagtgggtcggcttgatccgcgccaaggcgaacggcgatactgctgaatactcggccagcgtgaaggggcggttcaccatctcgagagatgacagcaagaactccctgtacctccaaatgaactccctgaaaaccgaggacactgcggtgtactactgcgcccgccagggtcgcggctacacgctggactattggggccagggcaccctggtcactgtgtcaagc

SEQ ID NO: 84 - DNA, 348 bp, Artificial Sequence
  source: /note="Description of Artificial Sequence: Synthetic polynucleotide"
caggtccaactgcagcagcctggggctgagcttgtgaagcctggggcttcagtgaagatgtcctgcaaggcttctggctacaccttcaccagctactggataacctgggtgaagcagaggcctggacaaggccttgagtggattggagatatttatcctggtagtggtagtactaactacaatgagaagttcaagagcaaggccacactgactgtagacacatcctccagcacagcctacatgcagctcagcagcctgacatctgaggactctgcggtctattactgtgcaagaggtagctactcccttgactactggggccaaggcaccactctcacagtctcctca

SEQ ID NO: 85 - DNA, 351 bp, Artificial Sequence
  source: /note="Description of Artificial Sequence: Synthetic polynucleotide"
gaggttcagctgcagcagtctgtggcagagcttgtgaggccaggggcctcagtcaagttgtcctgcacagcttctggcttcaacattaaaaacacctatatgcactgggtgaagcagaggcctgaacagggcctggagtggattggaaggattgatcctgcgaatggtaatactaaatatgccccgaagttccagggcaaggccactataactgcagacacatcctccaacacagcctacctgcagctcagcagcctgacatctgaggacactgccatctattactgtgctcctagtaactaccatgctatggactactggggtcaaggaacctcagtcaccgtctcctca

SEQ ID NO: 86 - DNA, 351 bp, Artificial Sequence
  source: /note="Description of Artificial Sequence: Synthetic polynucleotide"
gatgtacagcttcaggagtcaggacctggcctcgtgaaaccttctcagtctctgtctctcacctgctctgtcactggctactccatcaccagtggttattactggaactggatccggcagtttccaggaaacaaactggaatggatgggctacataagctacgatggtagcaataactacaacccatctctcaaaaatcgaatctccatcactcgtgacacatctaagaaccagtttttcctgaagttgaattctgtgactactgaggacacagccacatattactgtgcaagatggaatggtaactactttgactactggggccaaggcaccactctcacagtctcctca

SEQ ID NO: 87 - DNA, 360 bp, Artificial Sequence
  source: /note="Description of Artificial Sequence: Synthetic polynucleotide"
gaggtccagctgcaacagtctggacctgtgctggtgaagcctggggcttcagtgaagatgtcctgtaaggcttctggatacacattcactgactactatatgaactgggtgaagcagagccatggaaagagccttgagtggattggagttattaatccttacaacggtggtactagctacaaccagaagttcaagggcaaggccacattgactgttgacaagtcctccagcacagcctacatggagctcaacagcctgacatctgaggactctgcagtctattactgtgcaagaaccagacagctcgggctacgttggtttgcttactggggccaagggactctggtcactgtctctgca

SEQ ID NO: 88 - DNA, 336 bp, Artificial Sequence
  source: /note="Description of Artificial Sequence: Synthetic polynucleotide"
gatgttgtgatgacccaaactccactctccctgcctgtcagtcttggagatcaagcctccatctcttgcagatctagtcagagacttgtacacagtaatggaaacacctatttacattggtacctgcagaagccaggccagtctccaaagctcctgatctacaaagtttccaaccgattttctggggtcccagacaggttcagtggcagtggatcagggacagatttcacactcaagatcagcagagtggaggctgaggatctgggagtttatttctgctctcaaagtacacatgttccgtacacgttcggaggggggaccaagctggaaataaaa

SEQ ID NO: 89 - DNA, 321 bp, Artificial Sequence
  source: /note="Description of Artificial Sequence: Synthetic polynucleotide"
gacatccagatgactcagtccccgtcctcagtctccgcatccgtgggagatcgcgtgacgattacttgccgggcgtcgcagaacatcaacatctggctgtcgtggtaccagcagaagcccgggaaggctccgaagctgctgatctacaaggcctcaaacttgcacaccggcgtgccttcccgcttttctggttcgggctccgggactgacttcaccctgaccatcagcagcctgcaacccgaggacttcgccacctattactgcctccaaggacagtcctacccaagaaccttcggcggaggaaccaaggtcgaaatcaaa

SEQ ID NO: 90 - DNA, 336 bp, Artificial Sequence
  source: /note="Description of Artificial Sequence: Synthetic polynucleotide"
gatattgtgatgactcaggctgcaccctctgtacctgtcactcctggagagtcagtatccatctcctgcaggtctagtaagagtcttctgcatagtaatggcaacacttacttgtattggttcctgcagaggccaggccagtctcctcagcgcctgatatattatatgtccaaccttgcctcaggagtcccagacaggttcagtggcagagggtcaggaactgatttcacactgagaatcagtagagtggaggctgaggatgtgggtgtttattactgtatgcaaagtctagaatatcctctcacgttcggtgctgggaccaagctggagctgaaa

SEQ ID NO: 91 - DNA, 336 bp, Artificial Sequence
  source: /note="Description of Artificial Sequence: Synthetic polynucleotide"
gatattgtgatgactcaggctgcaccctctgtacctgtcactcctggagagtcagtatccatctcctgcaggtctagtaagagtctcctgcatagtaatggcaacacttacttgtattggttcctgcagaggccaggccagtctcctcagctcctgatatatcggatgtccaaccttgcctcaggagtcccagacaggttcagtggcagtgggtcaggaactgctttcacactgagaatcagtagagtggaggctgaggatgtgggtgtttattactgtatgcaacatctagaatatccgtacacgttcggaggggggaccaagctggaaataaaa

SEQ ID NO: 92 - DNA, 336 bp, Artificial Sequence
  source: /note="Description of Artificial Sequence: Synthetic polynucleotide"
gacattgtgatgtcacagtctccatcctccctggctgtgtcagcaggagagaaggtcactatgagctgcaaatccagtcagagtctgctcaacagtagaacccgaaagaactacttggcttggtaccagcagaaaccagggcagtctcctaaactgctgatctactgggcatccactagggaatctggggtccctgatcgcttcacaggcagtggatctgggacagatttcactctcaccatcagcagtgtgcaggctgaagacctggcagtttattactgcaagcaatcttataatctgtggacgttcggtggaggcaccaagctggaaatcaaa

SEQ ID NO: 93 - DNA, 321 bp, Artificial Sequence
  source: /note="Description of Artificial Sequence: Synthetic polynucleotide"
gacattcagatgacccagtctcctgcctcccagtctgcatctctgggagaaagtgtcaccatcacatgcctggcaagtcagaccattggtacatggttagcatggtatcagcagaaaccagggaaatctcctcagctcctgatttatgctgcaaccagcttggcagatggggtcccatcaaggttcagtggtagtggatctggcacaaaattttctttcaagatcagcagcctacaggctgaagattttgtaagttattactgtcaacaactttacagtactccgtggacgttcggtggaggcaccaagctggaaatcaaa

SEQ ID NO: 94 - protein, 23 aa, Artificial Sequence
  source: /note="Description of Artificial Sequence: Synthetic peptide"
GIGKHVGKALKGLKGLLKGLGES

SEQ ID NO: 95 - protein, 26 aa, Artificial Sequence
  source: /note="Description of Artificial Sequence: Synthetic peptide"
GRRKRKWLRRIGKGVKIIGGAALDHL

SEQ ID NO: 96 - protein, 27 aa, Artificial Sequence
  source: /note="Description of Artificial Sequence: Synthetic peptide"
GGLRSLGRKILRAWKKYGPQATPATRQ

SEQ ID NO: 97 - protein, 14 aa, Artificial Sequence
  source: /note="Description of Artificial Sequence: Synthetic peptide"
IKWKKLLRAAKRIL

SEQ ID NO: 98 - protein, 19 aa, Artificial Sequence
  source: /note="Description of Artificial Sequence: Synthetic peptide"
IGKKWKRIVKRIKKFLRKL

SEQ ID NO: 99 - protein, 12 aa, Artificial Sequence
  source: /note="Description of Artificial Sequence: Synthetic peptide"
ILGKIWKIKKLF

SEQ ID NO: 100 - protein, 37 aa, Artificial Sequence
  source: /note="Description of Artificial Sequence: Synthetic polypeptide"
RLGDILQKAREKIEGGLKKLVQKIKDFFGKFAPRTES

SEQ ID NO: 101 - protein, 30 aa, Artificial Sequence
  source: /note="Description of Artificial Sequence: Synthetic polypeptide"
GGGGRFKRFRKKFKKLFKKLSPVIPLLHLG

SEQ ID NO: 102 - protein, 27 aa, Artificial Sequence
  source: /note="Description of Artificial Sequence: Synthetic peptide"
GRFKRFRKKFKKLFKKLSPVIPLLHLG

SEQ ID NO: 103 - protein, 119 aa, Artificial Sequence
  source: /note="Description of Artificial Sequence: Synthetic polypeptide"
EVKLVESGGDLVKPGGSLRLSCAASEFTFSDYAMSWVRQTPAKRLEWVAYISSDGDSTYYPDNIKGRFTISRDNAKNTLYLQMNSLRSEDTAMYFCAREIRLRGYFDVWGAGTTVTVSS

SEQ ID NO: 104 - protein, 111 aa, Artificial Sequence
  source: /note="Description of Artificial Sequence: Synthetic polypeptide"
DIVLTQSPASLAVSLGQRATISCRASESVFGHGISPMHWYQQKPGQPPKLLIYRASNLKFGIPARFSGSGSRTDFTLTINPVEADDVATYYCQQSNEYPRTFGGGTKLEIK

SEQ ID NO: 105 - protein, 7 aa, Artificial Sequence
  source: /note="Description of Artificial Sequence: Synthetic peptide"
EFTFSDY

SEQ ID NO: 106 - protein, 6 aa, Artificial Sequence
  source: /note="Description of Artificial Sequence: Synthetic peptide"
SSDGDS

SEQ ID NO: 107 - protein, 10 aa, Artificial Sequence
  source: /note="Description of Artificial Sequence: Synthetic peptide"
EIRLRGYFDV

SEQ ID NO: 108 - protein, 5 aa, Artificial Sequence
  source: /note="Description of Artificial Sequence: Synthetic peptide"
DYAMS

SEQ ID NO: 109 - protein, 17 aa, Artificial Sequence
  source: /note="Description of Artificial Sequence: Synthetic peptide"
YISSDGDSTYYPDNIKG

SEQ ID NO: 110 - protein, 15 aa, Artificial Sequence
  source: /note="Description of Artificial Sequence: Synthetic peptide"
RASESVFGHGISPMH

SEQ ID NO: 111 - protein, 7 aa, Artificial Sequence
  source: /note="Description of Artificial Sequence: Synthetic peptide"
RASNLKF

SEQ ID NO: 112 - protein, 9 aa, Artificial Sequence
  source: /note="Description of Artificial Sequence: Synthetic peptide"
QQSNEYPRT

SEQ ID NO: 113 - DNA, 357 bp, Artificial Sequence
  source: /note="Description of Artificial Sequence: Synthetic polynucleotide"
gaagtgaagttggtggagtctgggggagacttggtgaaacctggagggtccctgagactctcctgtgcagcctctgaattcactttcagtgattatgccatgtcttgggttcgccagactccggcgaagaggctggagtgggtcgcatacattagtagtgatggtgatagtacctactatccggacaatattaagggccgattcaccatctccagagacaatgccaagaacaccctatacctgcaaatgaacagtctgaggtctgaggacacggccatgtatttttgtgcaagagaaatacggctaagggggtacttcgatgtctggggcgcagggaccacggtcaccgtctcctca

SEQ ID NO: 114 - DNA, 333 bp, Artificial Sequence
  source: /note="Description of Artificial Sequence: Synthetic polynucleotide"
gacattgtgctgacccaatctccagcttctttggctgtgtctctagggcagagggccaccatatcctgcagagccagtgaaagtgtttttggtcatggcattagtcctatgcactggtaccagcagaaaccaggacagccacccaaactcctcatctatcgtgcatccaacctaaaatttgggatccctgccaggttcagtggcagtgggtctaggacagacttcaccctcaccattaatcctgtggaggctgatgatgttgcaacctattactgtcagcaaagtaatgaatatcctcggacgttcggtggaggcaccaagctggagatcaaa

SEQ ID NO: 115 - protein, 119 aa, Artificial Sequence
  source: /note="Description of Artificial Sequence: Synthetic polypeptide"
EVKLVESGGGLVQPGGSLRLSCSASEFTFSDYAMSWVRQAPGKGLEWVSYISSDGDSTYYPDNIKGRFTISRDNSKNTLYVQMSSLRAEDTAVYFCAREIRLRGYFDVWGQGTTVTVSS

SEQ ID NO: 116 - protein, 119 aa, Artificial Sequence
  source: /note="Description of Artificial Sequence: Synthetic polypeptide"
EVKLVESGGGLVKPGGSLRLSCAASEFTFSDYAMSWVRQAPGKRLEWVAYISSDGDSIYYPDNIKGRFTISRDNAKNSLYLQMNSLRAEDTAMYFCAREIRLRGYFDVWGQGTTVTVSS

SEQ ID NO: 117 - protein, 119 aa, Artificial Sequence
  source: /note="Description of Artificial Sequence: Synthetic polypeptide"
EVKLVESGGGLVQPGGSLRLSCAASEFTFSDYAMSWVRQAPGKRLEWVAYISSDGDSTYYPDSVKGRFTISRDNAKNSLYLQMNSLRAEDTAMYFCAREIRLRGYFDVWGQGTTVTVSS

SEQ ID NO: 118 - protein, 119 aa, Artificial Sequence
  source: /note="Description of Artificial Sequence: Synthetic polypeptide"
EVKLVESGEGLVQPGGSLRLSCAASEFTFSDYAMSWVRQAPGKRLEWVAYISSDGDSTYYPDNIKGRFTISRDNSKNTLYLQMGSLRAEDMAMYFCAREIRLRGYFDVWGQGTTVTVSS

SEQ ID NO: 119 - protein, 111 aa, Artificial Sequence
  source: /note="Description of Artificial Sequence: Synthetic polypeptide"
EIVMTQSPATLSVSPGERATLSCRASESVFGHGISPLHWYQQKPGQAPKLLIYRASNRKTGIPARFSGSGSGTEFTLTISSLQSEDFAVYYCQQSNEYPRTFGGGTKVEIK

SEQ ID NO: 120 - protein, 111 aa, Artificial Sequence
  source: /note="Description of Artificial Sequence: Synthetic polypeptide"
DIQMTQSPSTLSASVGDRVTITCRASESVFGHGISPLHWYQQKPGKAPKLLIYRASNLKFGVPSRFSGSGSGTEFTLTISSLQPDDFATYYCQQSNEYPRTFGGGTKVEIK

SEQ ID NO: 121 - protein, 111 aa, Artificial Sequence
  source: /note="Description of Artificial Sequence: Synthetic polypeptide"
EIVMTQSPATLSVSPGERATLSCRASESVFGHGISPLHWYQQKPGQPPRLLIYRASNRKTGIPARFSGSGSGTEFTLTISSLQSEDFAVYYCQQSNEYPRTFGGGTKVEIK

SEQ ID NO: 122 - protein, 111 aa, Artificial Sequence
  source: /note="Description of Artificial Sequence: Synthetic polypeptide"
DIQMTQSPSTLSASVGDRVTITCRASESVFGHGISPLHWYQQKPGKAPKLLIYRASNLKFGVPSRFSGSGSRTDFTLTISSLQPDDFATYYCQQSNEYPRTFGGGTKVEIK

SEQ ID NO: 123 - protein, 111 aa, Artificial Sequence
  source: /note="Description of Artificial Sequence: Synthetic polypeptide"
DIQMTQSPSTLSASVGDRVTITCRASESVFGHGISPLHWYQQKPGKAPKLLIYRASNLKFGIPSRFSGSGSRTDFTLTISSLQPDDFATYYCQQSNEYPRTFGGGTKVEIK

SEQ ID NO: 124 - protein, 111 aa, Artificial Sequence
  source: /note="Description of Artificial Sequence: Synthetic polypeptide"
DIQMTQSPSTLSASVGDRVTITCRASESVFGHGISPLHWYQQKPGQPPKLLIYRASNLKFGIPSRFSGSGSGTEFTLTISSLQPDDFATYYCQQSNEYPRTFGGGTKVEIK

SEQ ID NO: 125 - protein, 111 aa, Artificial Sequence
  source: /note="Description of Artificial Sequence: Synthetic polypeptide"
DIVLTQSPSTLSASVGDRVTITCRASESVFGHGISPMHWYQQKPGKAPKLLIYRASNLKFGVPSRFSGSGSGTEFTLTISSLQPDDFATYYCQQSNEYPRTFGGGTKVEIK

SEQ ID NO: 126 - protein, 111 aa, Artificial Sequence
  source: /note="Description of Artificial Sequence: Synthetic polypeptide"
DIQMTQSPSTLSASVGDRVTITCRASESVFGHGISPLHWYQQKPGKAPKLLIYRASNLKFGIPARFSGSGSGTEFTLTISSLQPDDFATYYCQQSNEYPRTFGGGTKVEIK

SEQ ID NO: 127 - protein, 111 aa, Artificial Sequence
  source: /note="Description of Artificial Sequence: Synthetic polypeptide"
DIVLTQSPASLAVSLGQRATISCRASESIFGHGISPMHWYQQKPGQPPKLLIYRASNLKFGIPARFSGSGSRTDFTLTINPVEADDVATYYCQQSNEYPRTFGGGTKLEIK

SEQ ID NO: 128 - protein, 111 aa, Artificial Sequence
  source: /note="Description of Artificial Sequence: Synthetic polypeptide"
DIVLTQSPASLAVSLGQRATISCRASESVFGHGISPMHWYQQKPGQPPKLLIYRASSLKFGIPARFSGSGSRTDFTLTINPVEADDVATYYCQQSNEYPRTFGGGTKLEIK

SEQ ID NO: 129 - protein, 111 aa, Artificial Sequence
  source: /note="Description of Artificial Sequence: Synthetic polypeptide"
DIVLTQSPASLAVSLGQRATISCRASESVFGHGISPMHWYQQKPGQPPKLLIYRASNLKSGIPARFSGSGSRTDFTLTINPVEADDVATYYCQQSNEYPRTFGGGTKLEIK

SEQ ID NO: 130 - protein, 111 aa, Artificial Sequence
  source: /note="Description of Artificial Sequence: Synthetic polypeptide"
DIVMTQSPATLSVSPGERATLSCRASESVFGHGISPLHWYQQKPGQAPKLLIYRASNLKTGIPARFSGSGSRTDFTLTISSLQSEDFATYYCQQSNEYPRTFGGGTKVEIK

SEQ ID NO: 131 - protein, 111 aa, Artificial Sequence
  source: /note="Description of Artificial Sequence: Synthetic polypeptide"
EIVMTQSPATLSVSPGERATISCRASESVFGHGISPLHWYQQKPGQAPKLLIYRASNRKTGIPARFSGSGSGTEFTLTISPVQSEDFAVYYCQQSNEYPRTFGGGTKLEIK

SEQ ID NO: 132 - protein, 111 aa, Artificial Sequence
  source: /note="Description of Artificial Sequence: Synthetic polypeptide"
DIQMTQSPSTLSASVGDRVTITCRASESIFGHGISPLHWYQQKPGKAPKLLIYRASNLKSGIPSRFSGSGSRTEFTLTISSLQPDDFATYYCQQSNEYPRTFGGGTKVEIK

SEQ ID NO: 133 - protein, 111 aa, Artificial Sequence
  source: /note="Description of Artificial Sequence: Synthetic polypeptide"
DIQMTQSPSTLSASVGDRVTITCRASESIFGHGISPLHWYQQKPGKAPKLLIYRASNLKSGVPSRFSGSGSRTEFTLTISSLQPDDFATYYCQQSNEYPRTFGGGTKVEIK

SEQ ID NO: 134 - protein, 111 aa, Artificial Sequence
  source: /note="Description of Artificial Sequence: Synthetic polypeptide"
DIQMTQSPSTLSASVGDRVTITCRASESIFGHGISPLHWYQQKPGKAPKLLIYRASNLKSGVPARFSGSGSRTEFTLTISSLQPDDFATYYCQQSNEYPRTFGGGTKVEIK

SEQ ID NO: 135 - protein, 111 aa, Artificial Sequence
  source: /note="Description of Artificial Sequence: Synthetic polypeptide"
DIQMTQSPSTLSASVGDRVTITCRASESVFGHGISPLHWYQQKPGKAPKLLIYRASNLKSGVPSRFSGSGSRTEFTLTISSLQPDDFATYYCQQSNEYPRTFGGGTKVEIK

SEQ ID NO: 136 - protein, 111 aa, Artificial Sequence
  source: /note="Description of Artificial Sequence: Synthetic polypeptide"
DIQMTQSPSTLSASVGDRVTITCRASESIFGHGISPLHWYQQKPGKAPKLLIYRASNLKSGVPSRFSGSGSRTDFTLTISSLQPDDFATYYCQQSNEYPRTFGGGTKVEIK

SEQ ID NO: 137 - protein, 111 aa, Artificial Sequence
  source: /note="Description of Artificial Sequence: Synthetic polypeptide"
DIQMTQSPSTLSASVGDRVTITCRASESIFGHGISPLHWYQQKPGKAPKLLIYRASNLKSGIPSRFSGSGSRTDFTLTISSLQPDDFATYYCQQSNEYPRTFGGGTKVEIK

SEQ ID NO: 138 - protein, 15 aa, Artificial Sequence
  source: /note="Description of Artificial Sequence: Synthetic peptide"
RASESVFGHGISPLH

SEQ ID NO: 139 - protein, 7 aa, Artificial Sequence
  source: /note="Description of Artificial Sequence: Synthetic peptide"
RASNRKT

SEQ ID NO: 140 - protein, 15 aa, Artificial Sequence
  source: /note="Description of Artificial Sequence: Synthetic peptide"
RASESIFGHGISPMH

SEQ ID NO: 141 - protein, 7 aa, Artificial Sequence
  source: /note="Description of Artificial Sequence: Synthetic peptide"
RASSLKF

SEQ ID NO: 142 - protein, 7 aa, Artificial Sequence
  source: /note="Description of Artificial Sequence: Synthetic peptide"
RASNLKS

SEQ ID NO: 143 - protein, 7 aa, Artificial Sequence
  source: /note="Description of Artificial Sequence: Synthetic peptide"
RASNLKT

SEQ ID NO: 144 - protein, 15 aa, Artificial Sequence
  source: /note="Description of Artificial Sequence: Synthetic peptide"
RASESIFGHGISPLH

SEQ ID NO: 145 - protein, 17 aa, Artificial Sequence
  source: /note="Description of Artificial Sequence: Synthetic peptide"
YISSDGDSIYYPDNIKG

SEQ ID NO: 146 - protein, 17 aa, Artificial Sequence
  source: /note="Description of Artificial Sequence: Synthetic peptide"
YISSDGDSTYYPDSVKG

SEQ ID NO: 147 - protein, 40 aa, Artificial Sequence
  source: /note="Description of Artificial Sequence: Synthetic polypeptide"
GGGLLGDFFRKSKEKIGKEFKRIVQRIKDFLRNLVPRTES

SEQ ID NO: 148 - protein, 29 aa, Artificial Sequence
  source: /note="Description of Artificial Sequence: Synthetic peptide"
GGGKWKSFIKKLTKAAKKVVTTAKKPLIV

SEQ ID NO: 149 - protein, 18 aa, Artificial Sequence
  source: /note="Description of Artificial Sequence: Synthetic peptide"
GGGVNWKKILGKIIKVVK

SEQ ID NO: 150 - protein, 32 aa, Artificial Sequence
  source: /note="Description of Artificial Sequence: Synthetic polypeptide"
GGGTLISWIKNKRKQRPRVSRRRRRRGGRRRR

SEQ ID NO: 151 - protein, 29 aa, Artificial Sequence
  source: /note="Description of Artificial Sequence: Synthetic peptide"
GGGGIGAILKVLATGLPTLISWIKNKRKQ

SEQ ID NO: 152 - protein, 35 aa, Artificial Sequence
  source: /note="Description of Artificial Sequence: Synthetic polypeptide"
GGGGLRKRLRKFRNKIKEKLKKIGQKIQGLLPKLA

SEQ ID NO: 153 - protein, 31 aa, Artificial Sequence
  source: /note="Description of Artificial Sequence: Synthetic polypeptide"
GGGGLRRLGRKIAHGIKKYGPTILRIIRIAG

SEQ ID NO: 154 - protein, 32 aa, Artificial Sequence
  source: /note="Description of Artificial Sequence: Synthetic polypeptide"
GGGRGLRRLGRKIAHGVKKYGPTVLRIIKKYG

SEQ ID NO: 155 - protein, 37 aa, Artificial Sequence
  source: /note="Description of Artificial Sequence: Synthetic polypeptide"
GGGKRFKKFFKKLKNSVKKRAKKFFKKPRVIGVSIPF

SEQ ID NO: 156 - protein, 33 aa, Artificial Sequence
  source: /note="Description of Artificial Sequence: Synthetic polypeptide"
GGGKFFRKLKKSVKKRAKEFFKKPRVIGVSIPF

SEQ ID NO: 157 - protein, 30 aa, Artificial Sequence
  source: /note="Description of Artificial Sequence: Synthetic polypeptide"
GSGSGSGSGSGSGSGSGSGSGSGSGSGSGS

SEQ ID NO: 158 - protein, 22 aa, Artificial Sequence
  source: /note="Description of Artificial Sequence: Synthetic peptide"
GIGKFLKKAKKCGKACVKILKK

SEQ ID NO: 159 - protein, 30 aa, Artificial Sequence
  source: /note="Description of Artificial Sequence: Synthetic polypeptide"
GGGGRCKRFRKKCKKLFKKLSPVIPLLHLG

SEQ ID NO: 160 - protein, 5 aa, Staphylococcus aureus
  MOD_RES (3)..(3): Any amino acid
LPXTG

SEQ ID NO: 161 - protein, 5 aa, Staphylococcus pyogenes
  MOD_RES (3)..(3): Any amino acid
LPXTA

SEQ ID NO: 162 - protein, 5 aa, Staphylococcus sp.
LPETG

SEQ ID NO: 163 - protein, 25 aa, Artificial Sequence
  source: /note="Description of Artificial Sequence: Synthetic peptide"
GGGGIGKFLKKAKKFGKAFVKILKK

SEQ ID NO: 164 - protein, 11 aa, Artificial Sequence
  source: /note="Description of Artificial Sequence: Synthetic peptide"
  MOD_RES (4)..(4): D-Dab
  MOD_RES (5)..(6): Dab
  MISC_FEATURE (5)..(11): Cyclic
  MOD_RES (7)..(7): D-Leu
  MOD_RES (9)..(10): Dab
GGGXXXLFXXL

SEQ ID NO: 165 - protein, 17 aa, Artificial Sequence
  source: /note="Description of Artificial Sequence: Synthetic peptide"
  VARIANT (9)..(9): /replace="Thr"
  VARIANT (14)..(14): /replace="Ser"
  VARIANT (15)..(15): /replace="Val"
  MISC_FEATURE (1)..(17): /note="Variant residues given in the sequence have no preference with respect to those in the annotations for variant positions"
YISSDGDSIYYPDNIKG

SEQ ID NO: 166 - protein, 15 aa, Artificial Sequence
  source: /note="Description of Artificial Sequence: Synthetic peptide"
  VARIANT (6)..(6): /replace="Ile"
  VARIANT (14)..(14): /replace="Leu"
  MISC_FEATURE (1)..(15): /note="Variant residues given in the sequence have no preference with respect to those in the annotations for variant positions"
RASESVFGHGISPMH

SEQ ID NO: 167 - protein, 7 aa, Artificial Sequence
  source: /note="Description of Artificial Sequence: Synthetic peptide"
  VARIANT (4)..(4): /replace="Ser"
  VARIANT (5)..(5): /replace="Arg"
  VARIANT (7)..(7): /replace="Thr" or "Ser"
  MISC_FEATURE (1)..(7): /note="Variant residues given in the sequence have no preference with respect to those in the annotations for variant positions"
RASNLKF

SEQ ID NO: 168 - protein, 6 aa, Artificial Sequence
  source: /note="Description of Artificial Sequence: Synthetic peptide"
  MOD_RES (2)..(2): Formylglycine
LXTPSR

SEQ ID NO: 169 - protein, 6 aa, Artificial Sequence
  source: /note="Description of Artificial Sequence: Synthetic peptide"
LCTPSR

SEQ ID NO: 170 - protein, 7 aa, Artificial Sequence
  source: /note="Description of Artificial Sequence: Synthetic peptide"
AALLTGR

SEQ ID NO: 171 - protein, 7 aa, Artificial Sequence
  source: /note="Description of Artificial Sequence: Synthetic peptide"
SQLLTGR

SEQ ID NO: 172 - protein, 7 aa, Artificial Sequence
  source: /note="Description of Artificial Sequence: Synthetic peptide"
AAFMTGR

SEQ ID NO: 173 - protein, 7 aa, Artificial Sequence
  source: /note="Description of Artificial Sequence: Synthetic peptide"
AAFLTGR

SEQ ID NO: 174 - protein, 7 aa, Artificial Sequence
  source: /note="Description of Artificial Sequence: Synthetic peptide"
SAFLTGR

SEQ ID NO: 175 - protein, 7 aa, Artificial Sequence
  source: /note="Description of Artificial Sequence: Synthetic peptide"
ASILTGK

SEQ ID NO: 176 - protein, 7 aa, Artificial Sequence
  source: /note="Description of Artificial Sequence: Synthetic peptide"
VSFLTGR

SEQ ID NO: 177 - protein, 7 aa, Artificial Sequence
  source: /note="Description of Artificial Sequence: Synthetic peptide"
ASLLTGL

SEQ ID NO: 178 - protein, 7 aa, Artificial Sequence
  source: /note="Description of Artificial Sequence: Synthetic peptide"
ASILITG

SEQ ID NO: 179 - protein, 7 aa, Artificial Sequence
  source: /note="Description of Artificial Sequence: Synthetic peptide"
SAIMTGR

SEQ ID NO: 180 - protein, 7 aa, Artificial Sequence
  source: /note="Description of Artificial Sequence: Synthetic peptide"
SAIVTGR

SEQ ID NO: 181 - protein, 6 aa, Artificial Sequence
  source: /note="Description of Artificial Sequence: Synthetic peptide"
TNLWRG

SEQ ID NO: 182 - protein, 7 aa, Artificial Sequence
  source: /note="Description of Artificial Sequence: Synthetic peptide"
TNLWRGQ

SEQ ID NO: 183 - protein, 7 aa, Artificial Sequence
  source: /note="Description of Artificial Sequence: Synthetic peptide"
TNLCAAS

SEQ ID NO: 184 - protein, 7 aa, Artificial Sequence
  source: /note="Description of Artificial Sequence: Synthetic peptide"
VSLWTGK

SEQ ID NO: 185 - protein, 6 aa, Artificial Sequence
  source: /note="Description of Artificial Sequence: Synthetic peptide"
SMLLTG

SEQ ID NO: 186 - protein, 7 aa, Artificial Sequence
  source: /note="Description of Artificial Sequence: Synthetic peptide"
SMLLTGN

SEQ ID NO: 187 - protein, 7 aa, Artificial Sequence
  source: /note="Description of Artificial Sequence: Synthetic peptide"
SMLLTGT

SEQ ID NO: 188 - protein, 7 aa, Artificial Sequence
  source: /note="Description of Artificial Sequence: Synthetic peptide"
ASFMAGQ

SEQ ID NO: 189 - protein, 7 aa, Artificial Sequence
  source: /note="Description of Artificial Sequence: Synthetic peptide"
GSLFTGR

SEQ ID NO: 190 - protein, 7 aa, Artificial Sequence
  source: /note="Description of Artificial Sequence: Synthetic peptide"
  VARIANT (6)..(6): /replace="Ala"
  MISC_FEATURE (1)..(7): /note="Variant residues given in the sequence have no preference with respect to those in the annotations for variant positions"
CGPSRMS

SEQ ID NO: 191 - protein, 6 aa, Artificial Sequence
  source: /note="Description of Artificial Sequence: Synthetic peptide"
  VARIANT (6)..(6): /replace="Ala"
  MISC_FEATURE (1)..(6): /note="Variant residues given in the sequence have no preference with respect to those in the annotations for variant positions"
CGPSRM

SEQ ID NO: 192 - protein, 6 aa, Artificial Sequence
  source: /note="Description of Artificial Sequence: Synthetic peptide"
MCTPSR

SEQ ID NO: 193 - protein, 6 aa, Artificial Sequence
  source: /note="Description of Artificial Sequence: Synthetic peptide"
VCTPSR

SEQ ID NO: 194 - protein, 6 aa, Artificial Sequence
  source: /note="Description of Artificial Sequence: Synthetic peptide"
LCSPSR

SEQ ID NO: 195 - protein, 6 aa, Artificial Sequence
  source: /note="Description of Artificial Sequence: Synthetic peptide"
LCAPSR

SEQ ID NO: 196 - protein, 6 aa, Artificial Sequence
  source: /note="Description of Artificial Sequence: Synthetic peptide"
LCVPSR

SEQ ID NO: 197 - protein, 6 aa, Artificial Sequence
  source: /note="Description of Artificial Sequence: Synthetic peptide"
LCGPSR

SEQ ID NO: 198 - protein, 6 aa, Artificial Sequence
  source: /note="Description of Artificial Sequence: Synthetic peptide"
ICTPAR

SEQ ID NO: 199 - protein, 6 aa, Artificial Sequence
  source: /note="Description of Artificial Sequence: Synthetic peptide"
LCTPSK

SEQ ID NO: 200 - protein, 6 aa, Artificial Sequence
  source: /note="Description of Artificial Sequence: Synthetic peptide"
MCTPSK

SEQ ID NO: 201 - protein, 6 aa, Artificial Sequence
  source: /note="Description of Artificial Sequence: Synthetic peptide"
VCTPSK

SEQ ID NO: 202 - protein, 6 aa, Artificial Sequence
  source: /note="Description of Artificial Sequence: Synthetic peptide"
LCSPSK

SEQ ID NO: 203 - protein, 6 aa, Artificial Sequence
  source: /note="Description of Artificial Sequence: Synthetic peptide"
LCAPSK

SEQ ID NO: 204 - protein, 6 aa, Artificial Sequence
  source: /note="Description of Artificial Sequence: Synthetic peptide"
LCVPSK

SEQ ID NO: 205 - protein, 6 aa, Artificial Sequence
  source: /note="Description of Artificial Sequence: Synthetic peptide"
LCGPSK

SEQ ID NO: 206 - protein, 6 aa, Artificial Sequence
  source: /note="Description of Artificial Sequence: Synthetic peptide"
LCTPSA

SEQ ID NO: 207 - protein, 6 aa, Artificial Sequence
  source: /note="Description of Artificial Sequence: Synthetic peptide"
ICTPAA

SEQ ID NO: 208 - protein, 6 aa, Artificial Sequence
  source: /note="Description of Artificial Sequence: Synthetic peptide"
MCTPSA

SEQ ID NO: 209 - protein, 6 aa, Artificial Sequence
  source: /note="Description of Artificial Sequence: Synthetic peptide"
VCTPSA

SEQ ID NO: 210 - protein, 6 aa, Artificial Sequence
  source: /note="Description of Artificial Sequence: Synthetic peptide"
LCSPSA

SEQ ID NO: 211 - protein, 6 aa, Artificial Sequence
  source: /note="Description of Artificial Sequence: Synthetic peptide"
LCAPSA

SEQ ID NO: 212 - protein, 6 aa, Artificial Sequence
  source: /note="Description of Artificial Sequence: Synthetic peptide"
LCVPSA

SEQ ID NO: 213 - protein, 6 aa, Artificial Sequence
  source: /note="Description of Artificial Sequence: Synthetic peptide"
LCGPSA

SEQ ID NO: 214 - protein, 6 aa, Artificial Sequence
  source: /note="Description of Artificial Sequence: Synthetic peptide"
  MOD_RES (2)..(2): Formylglycine
LXTPSR

SEQ ID NO: 215 - protein, 6 aa, Artificial Sequence
  source: /note="Description of Artificial Sequence: Synthetic peptide"
  MOD_RES (2)..(2): Formylglycine
MXTPSR

SEQ ID NO: 216 - protein, 6 aa, Artificial Sequence
  source: /note="Description of Artificial Sequence: Synthetic peptide"
  MOD_RES (2)..(2): Formylglycine
VXTPSR

SEQ ID NO: 217 - protein, 6 aa, Artificial Sequence
  source: /note="Description of Artificial Sequence: Synthetic peptide"
  MOD_RES (2)..(2): Formylglycine
LXSPSR

SEQ ID NO: 218 - protein, 6 aa, Artificial Sequence
  source: /note="Description of Artificial Sequence: Synthetic peptide"
  MOD_RES (2)..(2): Formylglycine
LXAPSR

SEQ ID NO: 219 - protein, 6 aa, Artificial Sequence
  source: /note="Description of Artificial Sequence: Synthetic peptide"
  MOD_RES (2)..(2): Formylglycine
LXVPSR

SEQ ID NO: 220 - protein, 6 aa, Artificial Sequence
  source: /note="Description of Artificial Sequence: Synthetic peptide"
  MOD_RES (2)..(2): Formylglycine
LXGPSR

SEQ ID NO: 221 - protein, 6 aa, Artificial Sequence
  source: /note="Description of Artificial Sequence: Synthetic peptide"
  MOD_RES (2)..(2): Formylglycine
IXTPAR

SEQ ID NO: 222 - protein, 6 aa, Artificial Sequence
  source: /note="Description of Artificial Sequence: Synthetic peptide"
  MOD_RES (2)..(2): Formylglycine
LXTPSK

SEQ ID NO: 223 - protein, 6 aa, Artificial Sequence
  source: /note="Description of Artificial Sequence: Synthetic peptide"
  MOD_RES (2)..(2): Formylglycine
MXTPSK

SEQ ID NO: 224 - protein, 6 aa, Artificial Sequence
  source: /note="Description of Artificial Sequence: Synthetic peptide"
  MOD_RES (2)..(2): Formylglycine
VXTPSK

SEQ ID NO: 225 - protein, 6 aa, Artificial Sequence
  source: /note="Description of Artificial Sequence: Synthetic peptide"
  MOD_RES (2)..(2): Formylglycine
LXSPSK

SEQ ID NO: 226 - protein, 6 aa, Artificial Sequence
  source: /note="Description of Artificial Sequence: Synthetic peptide"
  MOD_RES (2)..(2): Formylglycine
LXAPSK

SEQ ID NO: 227 - protein, 6 aa, Artificial Sequence
  source: /note="Description of Artificial Sequence: Synthetic peptide"
  MOD_RES (2)..(2): Formylglycine
LXVPSK

SEQ ID NO: 228 - protein, 6 aa, Artificial Sequence
  source: /note="Description of Artificial Sequence: Synthetic peptide"
  MOD_RES (2)..(2): Formylglycine
LXGPSK

SEQ ID NO: 229 - protein, 6 aa, Artificial Sequence
  source: /note="Description of Artificial Sequence: Synthetic peptide"
  MOD_RES (2)..(2): Formylglycine
LXTPSA

SEQ ID NO: 230 - protein, 6 aa, Artificial Sequence
  source: /note="Description of Artificial Sequence: Synthetic peptide"
  MOD_RES (2)..(2): Formylglycine
MXTPSA

SEQ ID NO: 231 - protein, 6 aa, Artificial Sequence
  source: /note="Description of Artificial Sequence: Synthetic peptide"
  MOD_RES (2)..(2): Formylglycine
VXTPSA

SEQ ID NO: 232 - protein, 6 aa, Artificial Sequence
  source: /note="Description of Artificial Sequence: Synthetic peptide"
  MOD_RES (2)..(2): Formylglycine
LXSPSA

SEQ ID NO: 233 - protein, 6 aa, Artificial Sequence
  source: /note="Description of Artificial Sequence: Synthetic peptide"
  MOD_RES (2)..(2): Formylglycine
LXAPSA

SEQ ID NO: 234 - protein, 6 aa, Artificial Sequence
  source: /note="Description of Artificial Sequence: Synthetic peptide"
  MOD_RES (2)..(2): Formylglycine
LXVPSA

SEQ ID NO: 235 - protein, 6 aa, Artificial Sequence
  source: /note="Description of Artificial Sequence: Synthetic peptide"
  MOD_RES (2)..(2): Formylglycine
LXGPSA

SEQ ID NO: 236 - protein, 5 aa, Artificial Sequence
  source: /note="Description of Artificial Sequence: Synthetic peptide"
GSGGS

SEQ ID NO: 237 - protein, 4 aa, Artificial Sequence
  source: /note="Description of Artificial Sequence: Synthetic peptide"
GGGS

SEQ ID NO: 238 - protein, 5 aa, Artificial Sequence
  source: /note="Description of Artificial Sequence: Synthetic peptide"
GGSGG

SEQ ID NO: 239 - protein, 5 aa, Artificial Sequence
  source: /note="Description of Artificial Sequence: Synthetic peptide"
GSGSG

SEQ ID NO: 240 - protein, 5 aa, Artificial Sequence
  source: /note="Description of Artificial Sequence: Synthetic peptide"
GSGGG

SEQ ID NO: 241 - protein, 5 aa, Artificial Sequence
  source: /note="Description of Artificial Sequence: Synthetic peptide"
GGGSG

SEQ ID NO: 242 - protein, 5 aa, Artificial Sequence
  source: /note="Description of Artificial Sequence: Synthetic peptide"
GSSSG

SEQ ID NO: 243 - protein, 16 aa, Artificial Sequence
  source: /note="Description of Artificial Sequence: Synthetic peptide"
LCTPSRGGGGLCTPSR

SEQ ID NO: 244 - protein, 7 aa, Unknown
  source: /note="Description of Unknown: Sortase A recognition sequence"
LPETGGG

SEQ ID NO: 245 - protein, 22 aa, Artificial Sequence
  source: /note="Description of Artificial Sequence: Synthetic peptide"
GIGKFLKKAKKFGKAFVKILKK

SEQ ID NO: 246 - protein, 33 aa, Artificial Sequence
  source: /note="Description of Artificial Sequence: Synthetic polypeptide"
GGGKFFRALKKSVAKRAKEFFKAPRVIGVSIPF

SEQ ID NO: 247 - protein, 33 aa, Artificial Sequence
  source: /note="Description of Artificial Sequence: Synthetic polypeptide"
GGGKFFRTLKKSVTKRAKEFFKTPRVIGVSIPF

SEQ ID NO: 248 - protein, 33 aa, Artificial Sequence
  source: /note="Description of Artificial Sequence: Synthetic polypeptide"
GGGKFFRTLKKSVKTRAKEFFKTPRVIGVSIPF

SEQ ID NO: 249 - protein, 33 aa, Artificial Sequence
  source: /note="Description of Artificial Sequence: Synthetic polypeptide"
GGGKFFAKLKKSVKKRAKEFFKKPAVIGVSIPF

SEQ ID NO: 250 - protein, 33 aa, Artificial Sequence
  source: /note="Description of Artificial Sequence: Synthetic polypeptide"
GGGKFFAKLKKSVKKRAKEFFAKPRVIGVSIPF

SEQ ID NO: 251 - protein, 33 aa, Artificial Sequence
  source: /note="Description of Artificial Sequence: Synthetic polypeptide"
GGGKFFSKLKKSVKKRAKEFFSKPRVIGVSIPF

SEQ ID NO: 252 - protein, 33 aa, Artificial Sequence
  source: /note="Description of Artificial Sequence: Synthetic polypeptide"
GGGAFFAKLKKSVKKRAKEFFKKPRVIGVSIPF

SEQ ID NO: 253 - protein, 33 aa, Artificial Sequence
  source: /note="Description of Artificial Sequence: Synthetic polypeptide"
GGGKFFRKLKKSVKKRAKEFFAKPAVIGVSIPF

SEQ ID NO: 254 - protein, 41 aa, Artificial Sequence
  source: /note="Description of Artificial Sequence: Synthetic polypeptide"
GGGEEEEAAAGKFFRKLKKSVKKRAKEFFKKPRVIGVSIPF

SEQ ID NO: 255 - protein, 41 aa, Artificial Sequence
  source: /note="Description of Artificial Sequence: Synthetic polypeptide"
GGGKFFRKLKKSVKKRAKEFFKKPRVIGVSIPFAAAGEEEE

SEQ ID NO: 256 - protein, 44 aa, Artificial Sequence
  source: /note="Description of Artificial Sequence: Synthetic polypeptide"
GGGKFFRKLKKSVKKRAKEFFKKPRVIGVSIPFAAAGAVEDLED

SEQ ID NO: 257 - protein, 49 aa, Artificial Sequence
  source: /note="Description of Artificial Sequence: Synthetic polypeptide"
NRGECPGGGGSGSGSGSGSGSGSGSGSGSGSGSGSGSGSASLPETGGSG

SEQ ID NO: 258 - protein, 43 aa, Artificial Sequence
  source: /note="Description of Artificial Sequence: Synthetic polypeptide"
PGKGSGSGSGSGSGSGSGSGSGSGSGSGSGSGSASLPETGGSG

SEQ ID NO: 259 - protein, 6 aa, Artificial Sequence
  source: /note="Description of Artificial Sequence: Synthetic 6xHis tag"
HHHHHH

SEQ ID NO: 260 - protein, 5 aa, Unknown
  source: /note="Description of Unknown: Sortase A recognition sequence"
  MOD_RES (3)..(3): Any amino acid
LPXTG

SEQ ID NO: 261 - protein, 7 aa, Unknown
  source: /note="Description of Unknown: Sortase A recognition sequence"
  MOD_RES (3)..(3): Any amino acid
LPXTGGG